European Patent Specification EP 3 517 125 B1, published May 31, 2023. Title: CHIMERIC ANTIGEN RECEPTOR FOR EFFICIENT SELECTIVE PROLIFERATION IN VITRO AND USES THEREOF. Applicant: Xuanwu Hospital Of Capital Medical University. The sequence listing filed with the application follows.

SEQUENCE LISTING (14 sequences)

SEQ ID NO: 1 - DNA, 63 bp, Homo sapiens
atggcgctgccggtgaccgcgctgctgctgccgctggcgctgctgctgcatgcggcgcgtccg

SEQ ID NO: 2 - DNA, 207 bp, Artificial Sequence
accaccaccccggcgccgcgtccgccgaccccggcgccgaccattgcgagccagccgctgagcctgcgtccggaagcgtgccgtccggcggcgggcggcgcggtgcatacccgtggcctggattttgcgtgcgatatttatatttgggcgccgctggcgggcacctgcggcgtgctgctgctgagcctggtgattaccctgtattgc

SEQ ID NO: 3 - DNA, 462 bp, Artificial Sequence
aaacgtggccgtaaaaaactgctgtatatttttaaacagccgtttatgcgtccggtgcagaccacccaggaagaagatggctgcagctgccgttttccggaagaagaagaaggcggctgcgaactgcgtgtgaaatttagccgtagcgcggatgcgccggcgtataaacagggccagaaccagctgtataacgaactgaacctgggccgtcgtgaagaatatgatgtgctggataaacgtcgtggccgtgatccggaaatgggcggcaaaccgcgtcgtaaaaacccgcaggaaggcctgtataacgaactgcagaaagataaaatggcggaagcgtatagcgaaattggcatgaaaggcgaacgtcgtcgtggcaaaggccatgatggcctgtatcagggcctgagcaccgcgaccaaagatacctatgatgcgctgcatatgcaggcgctgccgccgcgt

SEQ ID NO: 4 - DNA, 30 bp, Homo sapiens
aaaccgctgccggaagtgaccgatgaatat

SEQ ID NO: 5 - DNA, 372 bp, Artificial Sequence
caggtgcagctgcagcagagcggcgcggaactggtgcgtccgggcagcagcgtgaaaattagctgcaaagcgagcggctatgcgtttagcagctattggatgaactgggtgaaacagcgtccgggccagggcctggaatggattggccagatttggccgggcgatggcgataccaactataacggcaaatttaaaggcaaagcgaccctgaccgcggatgaaagcagcagcaccgcgtatatgcagctgagcagcctggcgagcgaagatagcgcggtgtatttttgcgcgcgtcgtgaaaccaccaccgtgggccgttattattatgcgatggattattggggccagggcaccaccgtgaccgtgagcagc

SEQ ID NO: 6 - DNA, 333 bp, Artificial Sequence
gatattcagctgacccagagcccggcgagcctggcggtgagcctgggccagcgtgcgaccattagctgcaaagcgagccagagcgtggattatgatggcgatagctatctgaactggtatcagcagattccgggccagccgccgaaactgctgatttatgatgcgagcaacctggtgagcggcattccgccgcgttttagcggcagcggcagcggcaccgattttaccctgaacattcatccggtggaaaaagtggatgcggcgacctatcattgccagcagagcaccgaagatccgtggacctttggcggcggcaccaaactggaaattaaa

SEQ ID NO: 7 - DNA, 1500 bp, Artificial Sequence
atggctctgccagtgacagctctgctgctgcctctggctctgctgctgcacgcagctagaccccaggtgcagctgcagcagtcaggagcagaactcgtgagaccaggcagcagcgtgaagatctcttgcaaggccagcggctacgccttctctagctattggatgaattgggtgaagcagcggccaggacagggactggagtggattggacagatttggcccggcgacggcgataccaactacaacggcaagttcaagggcaaggccaccctgacagccgacgagtctagcagcacagcctacatgcagctgagctctctggccagcgaggatagcgccgtgtacttttgcgccagaagggagaccacaacagtgggccggtactactacgccatggactattggggccagggcacaaccgtgacagtgtctagcggaggaggcggctctaagcctctgccagaagtgacagacgagtacggcggaggaggaagcgacatccagctgacccagagcccagcttctctggcagtgtctctgggacagagggctaccatctcttgcaaggccagccagagcgtggattacgacggcgacagctacctgaattggtatcagcagatccccggccagcctcctaagctgctgatctacgacgcctccaacctggtgtccggcatccctcccagattcagcggaagcggcagcggcacagacttcaccctgaacatccaccccgtggagaaggtggacgccgccacataccattgccagcagagcacagaggacccctggacctttggcggcggaacaaagctggagatcaagacaaccaccccagcccctagacctcctacaccagcccctacaatcgcctctcagcctctgagcctgaggccagaagcttgtagacccgcagcaggaggagcagtgcatacaaggggcctggacttcgcttgcgacatctacatttgggcccctctggcaggaacttgcggagtgctgctgctgtctctggtcatcaccctgtattgcaagcggggccggaagaagctgctgtacatcttcaagcagcccttcatgcggccagtgcagacaacacaggaggaggacggttgcagctgcagattcccagaggaggaggaaggcggctgcgagctgagagtgaagttcagcaggagcgccgacgctccagcctataaacagggacagaaccagctgtacaacgagctgaacctgggcagaagagaggagtacgacgtgctggacaagaggagaggcagagacccagagatgggcggcaagcctagaaggaagaacccccaggagggcctgtacaacgagctgcagaaggacaagatggccgaggcttacagcgagatcggcatgaagggcgagaggagaagaggcaaaggccacgacggactgtatcagggactgagcacagccaccaaggacacctacgacgctctgcacatgcaggctctgcctcctagataa

SEQ ID NO: 8 - protein, 499 aa, Artificial Sequence
MALPVTALLLPLALLLHAARPQVQLQQSGAELVRPGSSVKISCKASGYAFSSYWMNWVKQRPGQGLEWIGQIWPGDGDTNYNGKFKGKATLTADESSSTAYMQLSSLASEDSAVYFCARRETTTVGRYYYAMDYWGQGTTVTVSSGGGGSKPLPEVTDEYGGGGSDIQLTQSPASLAVSLGQRATISCKASQSVDYDGDSYLNWYQQIPGQPPKLLIYDASNLVSGIPPRFSGSGSGTDFTLNIHPVEKVDAATYHCQQSTEDPWTFGGGTKLEIKTTTPAPRPPTPAPTIASQPLSLRPEACRPAAGGAVHTRGLDFACDIYIWAPLAGTCGVLLLSLVITLYCKRGRKKLLYIFKQPFMRPVQTTQEEDGCSCRFPEEEEGGCELRVKFSRSADAPAYKQGQNQLYNELNLGRREEYDVLDKRRGRDPEMGGKPRRKNPQEGLYNELQKDKMAEAYSEIGMKGERRRGKGHDGLYQGLSTATKDTYDALHMQALPPR

SEQ ID NO: 9 - protein, 263 aa, Artificial Sequence
MALPVTALLLPLALLLHAARPDIQMTQTTSSLSASLGDRVTISCRASQDISKYLNWYQQKPDGTVKLLIYHTSRLHSGVPSRFSGSGSGTDYSLTISNLEQEDIATYFCQQGNTLPYTFGGGTKLEITGGGGSGGGGSGGGGSEVKLQESGPGLVAPSQSLSVTCTVSGVSLPDYGVSWIRQPPRKGLEWLGVIWGSETTYYNSALKSRLTIIKDNSKSQVFLKMNSLQTDDTAIYYCAKHYYYGGSYAMDYWGQGTSVTVSS

SEQ ID NO: 10 - protein, 10 aa, Artificial Sequence
GGGGSGGGGS

SEQ ID NO: 11 - DNA, 15 bp, Artificial Sequence
ggcggcggcggcagc

SEQ ID NO: 12 - protein, 497 aa, Artificial Sequence
MALPVTALLLPLALLLHAARPQVQLQQSGAELVRPGSSVKISCKASGYAFSSYWMNWVKQRPGQGLEWIGQIWPGDGDTNYNGKFKGKATLTADESSSTAYMQLSSLASEDSAVYFCARRETTTVGRYYYAMDYWGQGTTVTVSSGGGGSWSHPQFEKGGGGSDIQLTQSPASLAVSLGQRATISCKASQSVDYDGDSYLNWYQQIPGQPPKLLIYDASNLVSGIPPRFSGSGSGTDFTLNIHPVEKVDAATYHCQQSTEDPWTFGGGTKLEIKTTTPAPRPPTPAPTIASQPLSLRPEACRPAAGGAVHTRGLDFACDIYIWAPLAGTCGVLLLSLVITLYCKRGRKKLLYIFKQPFMRPVQTTQEEDGCSCRFPEEEEGGCELRVKFSRSADAPAYKQGQNQLYNELNLGRREEYDVLDKRRGRDPEMGGKPRRKNPQEGLYNELQKDKMAEAYSEIGMKGERRRGKGHDGLYQGLSTATKDTYDALHMQALPPR

SEQ ID NO: 13 - protein, 498 aa, Artificial Sequence
MALPVTALLLPLALLLHAARPQVQLQQSGAELVRPGSSVKISCKASGYAFSSYWMNWVKQRPGQGLEWIGQIWPGDGDTNYNGKFKGKATLTADESSSTAYMQLSSLASEDSAVYFCARRETTTVGRYYYAMDYWGQGTTVTVSSGGGGSNWSHPQFEKGGGGSDIQLTQSPASLAVSLGQRATISCKASQSVDYDGDSYLNWYQQIPGQPPKLLIYDASNLVSGIPPRFSGSGSGTDFTLNIHPVEKVDAATYHCQQSTEDPWTFGGGTKLEIKTTTPAPRPPTPAPTIASQPLSLRPEACRPAAGGAVHTRGLDFACDIYIWAPLAGTCGVLLLSLVITLYCKRGRKKLLYIFKQPFMRPVQTTQEEDGCSCRFPEEEEGGCELRVKFSRSADAPAYKQGQNQLYNELNLGRREEYDVLDKRRGRDPEMGGKPRRKNPQEGLYNELQKDKMAEAYSEIGMKGERRRGKGHDGLYQGLSTATKDTYDALHMQALPPR

SEQ ID NO: 14 - DNA, 24 bp, Artificial Sequence
tggagccatccgcagtttgaaaaa